European Patent Specification EP 4 326 717 B1, published April 16, 2025. Title: Modified Ferroportin Inhibitors. Applicant: Vifor (International) AG. The sequence listing filed with the application follows.

SEQUENCE LISTING (2 sequences)

SEQ ID NO: 1 - DNA, 21 bp, human
  forward primer
caggtttgtgagcatcctgaa

SEQ ID NO: 2 - DNA, 19 bp, human
  reverse primer
ggcggcgactaaggagagg